European Patent Application EP 4 353 267 A1, published April 17, 2024. Title: A conjugated antibody liposome. Applicant: Hangzhou HighField BioPharmaceuticals Corporation. The sequence listing filed with the application follows.

SEQUENCE LISTING (4 sequences)

SEQ ID NO: 1 - protein, 231 aa, Artificial Sequence
  aHER2 Fab Heavy chain
EVQLVESGGGLVQPGGSLRLSCAASGFNIKDTYIHWVRQAPGKGLEWVARIYPTNGYTRYADSVKGRFTISADTSKNTAYLQMNSLRAEDTAVYYCSRWGGDGFYAMDYWGQGTLVTVSSASTKGPSVFPLAPSSKSTSGGTAALGCLVKDYFPEPVTVSWNSGALTSGVHTFPAVLQSSGLYSLSSVVTVPSSSLGTQTYICNVNHKPSNTKVDKKVEPKSCDKTHTCAA

SEQ ID NO: 2 - protein, 214 aa, Artificial Sequence
  aHER2 Fab Light chain
DIQMTQSPSSLSASVGDRVTITCRASQDVNTAVAWYQQKPGKAPKLLIYSASFLYSGVPSRFSGSRSGTDFTLTISSLQPEDFATYYCQQHYTTPPTFGQGTKVEIKRTVAAPSVFIFPPSDEQLKSGTASVVCLLNNFYPREAKVQWKVDNALQSGNSQESVTEQDSKDSTYSLSSTLTLSKADYEKHKVYACEVTHQGLSSPVTKSFNRGEC

SEQ ID NO: 3 - protein, 233 aa, Artificial Sequence
  aCD3 Fab Heavy chain
EVQLVESGGGLVQPGGSLRLSCAASGYSFTGYTMNWVRQAPGKGLEWVALINPYKGVTTYADSVKGRFTISVDKSKNTAYLQMNSLRAEDTAVYYCARSGYYGDSDWYFDVWGQGTLVTVSSASTKGPSVFPLAPSSKSTSGGTAALGCLVKDYFPEPVTVSWNSGALTSGVHTFPAVLQSSGLYSLSSVVTVPSSSLGTQTYICNVNHKPSNTKVDKKVEPKSCDKTHTCAA

SEQ ID NO: 4 - protein, 214 aa, Artificial Sequence
  aCD3 Fab Light chain
DIQMTQSPSSLSASVGDRVTITCRASQDIRNYLNWYQQKPGKAPKLLIYYTSRLESGVPSRFSGSGSGTDYTLTISSLQPEDFATYYCQQGNTLPWTFGQGTKVEIKRTVAAPSVFIFPPSDEQLKSGTASVVCLLNNFYPREAKVQWKVDNALQSGNSQESVTEQDSKDSTYSLSSTLTLSKADYEKHKVYACEVTHQGLSSPVTKSFNRGEC